European Patent Specification EP 3 445 393 B1, published January 14, 2026. Title: CMV Neutralizing Antigen Binding Proteins. Applicant: FU, TONG-MING TANG, AIMIN WANG, DAI AN, ZHIQIANG ZHANG, NINGYAN HA, SHA. Application 62/324952. The sequence listing filed with the application follows.

SEQUENCE LISTING (149 sequences)

SEQ ID NO: 1 - protein, 8 aa, Homo sapiens
GFSFSDHD

SEQ ID NO: 2 - protein, 10 aa, Homo sapiens
SRNKDYSSTT

SEQ ID NO: 3 - protein, 19 aa, Homo sapiens
ARGPHHSDRSGYYGGTFDI

SEQ ID NO: 4 - protein, 6 aa, Homo sapiens
QGISSW

SEQ ID NO: 5 - protein, 3 aa, Homo sapiens
DAS

SEQ ID NO: 6 - protein, 9 aa, Homo sapiens
QQGNMFPLT

SEQ ID NO: 7 - protein, 8 aa, Homo sapiens
GYTFTNYA

SEQ ID NO: 8 - protein, 8 aa, Homo sapiens
INAGRGNT

SEQ ID NO: 9 - protein, 15 aa, Homo sapiens
ARDESTGDYYYYMDV

SEQ ID NO: 10 - protein, 6 aa, Homo sapiens
RLDDKY

SEQ ID NO: 11 - protein, 3 aa, Homo sapiens
QDN

SEQ ID NO: 12 - protein, 9 aa, Homo sapiens
QAWDSDTYV

SEQ ID NO: 13 - protein, 8 aa, Homo sapiens
EFTFSDYY

SEQ ID NO: 14 - protein, 8 aa, Homo sapiens
ISSSGTTI

SEQ ID NO: 15 - protein, 19 aa, Homo sapiens
ARDSYSKLVDIEAIEAFDI

SEQ ID NO: 16 - protein, 6 aa, Homo sapiens
NIGSKS

SEQ ID NO: 17 - protein, 3 aa, Homo sapiens
FDT

SEQ ID NO: 18 - protein, 11 aa, Homo sapiens
QVWDRTSDHVV

SEQ ID NO: 19 - protein, 8 aa, Homo sapiens
GFTFSDYY

SEQ ID NO: 20 - protein, 8 aa, Homo sapiens
ISSSGRTI

SEQ ID NO: 21 - protein, 6 aa, Homo sapiens
NIGGKS

SEQ ID NO: 22 - protein, 3 aa, Homo sapiens
YDS

SEQ ID NO: 23 - protein, 11 aa, Homo sapiens
QVWDRHGDHVV

SEQ ID NO: 24 - protein, 8 aa, Homo sapiens
GFNFKDYY

SEQ ID NO: 25 - protein, 8 aa, Homo sapiens
ISSSGQTI

SEQ ID NO: 26 - protein, 19 aa, Homo sapiens
ARDSYSKLVDIVAIEAFDL

SEQ ID NO: 27 - protein, 11 aa, Homo sapiens
QVWDSSSARLV

SEQ ID NO: 28 - protein, 8 aa, Homo sapiens
GFSFSAYY

SEQ ID NO: 29 - protein, 8 aa, Homo sapiens
ISSSGNTI

SEQ ID NO: 30 - protein, 19 aa, Homo sapiens
ARDSYSKLADIEATEAFDV

SEQ ID NO: 31 - protein, 11 aa, Homo sapiens
QVWDSGSDRVV

SEQ ID NO: 32 - protein, 8 aa, Homo sapiens
ISGSGRTL

SEQ ID NO: 33 - protein, 19 aa, Homo sapiens
ARDSYSKLVEIEAIEAFDV

SEQ ID NO: 34 - protein, 11 aa, Homo sapiens
QVWDRQTDHVV

SEQ ID NO: 35 - protein, 10 aa, Homo sapiens
GDAISGSNYY

SEQ ID NO: 36 - protein, 7 aa, Homo sapiens
IYHTGST

SEQ ID NO: 37 - protein, 12 aa, Homo sapiens
ARRIRGYSGTYD

SEQ ID NO: 38 - protein, 6 aa, Homo sapiens
QDISSY

SEQ ID NO: 39 - protein, 3 aa, Homo sapiens
SAS

SEQ ID NO: 40 - protein, 5 aa, Homo sapiens
QQLNN

SEQ ID NO: 41 - protein, 8 aa, Homo sapiens
GFAFDNYA

SEQ ID NO: 42 - protein, 8 aa, Homo sapiens
ISLEGRNK

SEQ ID NO: 43 - protein, 22 aa, Homo sapiens
ARDMRYYYDSNGHYRNRYGMDV

SEQ ID NO: 44 - protein, 6 aa, Homo sapiens
QDINQF

SEQ ID NO: 45 - protein, 8 aa, Homo sapiens
QQYENLFT

SEQ ID NO: 46 - protein, 8 aa, Homo sapiens
GYTFNTYA

SEQ ID NO: 47 - protein, 8 aa, Homo sapiens
INTYSGST

SEQ ID NO: 48 - protein, 12 aa, Homo sapiens
ARDGYNWGFLDF

SEQ ID NO: 49 - protein, 6 aa, Homo sapiens
QGISNY

SEQ ID NO: 50 - protein, 3 aa, Homo sapiens
AAS

SEQ ID NO: 51 - protein, 9 aa, Homo sapiens
QKYNSAPLT

SEQ ID NO: 52 - protein, 8 aa, Homo sapiens
GYRFTIYS

SEQ ID NO: 53 - protein, 8 aa, Homo sapiens
INTYNGNT

SEQ ID NO: 54 - protein, 12 aa, Homo sapiens
ARDAENWGFFDD

SEQ ID NO: 55 - protein, 6 aa, Homo sapiens
QSVGRH

SEQ ID NO: 56 - protein, 3 aa, Homo sapiens
GAS

SEQ ID NO: 57 - protein, 9 aa, Homo sapiens
QQYNTWPYT

SEQ ID NO: 58 - protein, 8 aa, Homo sapiens
GFTFSNHG

SEQ ID NO: 59 - protein, 8 aa, Homo sapiens
VSKDGTNE

SEQ ID NO: 60 - protein, 18 aa, Homo sapiens
AREGYCGDDRCYSGQPDY

SEQ ID NO: 61 - protein, 6 aa, Homo sapiens
QSVGRY

SEQ ID NO: 62 - protein, 3 aa, Homo sapiens
DSS

SEQ ID NO: 63 - protein, 10 aa, Homo sapiens
QQRSHWPPLT

SEQ ID NO: 64 - DNA, 384 bp, Homo sapiens
gaggtgcaactggtgcagtctgggggaggcttggtccagcctggagggtccctgagagtctcctgtgcagcctctggattcagcttcagtgaccacgacatggactgggtccgccaggctccagggaaggggtttgagtgggtcggccgtagcagaaacaaagattacagttccaccacagaatatgccgcgtctgtgaggggcagattcaccatctcaagacatacttcagaggatttactgtatctggagttgaacaccgtgaaaaccgaggacacggccgtgtatttttgtgctagaggacctcatcactctgatcggagtggttattacgggggaacttttgatatctggggccaagggaccatggtcaccgtgtcctca

SEQ ID NO: 65 - DNA, 366 bp, Homo sapiens
caagtgcagctcgtggagtctggggctgaggtgaagaagcctggggccttagtgaaggtttcctgcaaggcttctggatacaccttcactaactatgctatacattgggtgcgccaggcctccggacaaaggcttgagtggatgggatggatcaacgctggcagaggtaacacaaaatattcacagaagttccagggcagagtcaccattactagggacacatccgcgagcacagcctacatggagctgagcagtttgagatctgaggacgcggctgtttatttctgtgcgagagatgagtcaactggtgactactactactacatggacgtctggggcaaagggaccacggtcaccgtctcttca

SEQ ID NO: 66 - DNA, 378 bp, Homo sapiens
caggtgcagctggtggcgtctgggggaggcttggtcaagcctggcgggtccctgagactctcctgtgcagcctctgaattcaccttcagtgactactacatgacctggatccgccaggctccagggaaggggctggagtgggtctcgtatattagtagtagtggtacgaccatatactacgccgactctgtgaagggccgattcaccgtctccagggacaacgccaagaactcactgtttctgcaaatgaacagcctgagagccgaggacacggctctttattattgtgcgagagactcttattcgaagttggtggatatagaggccatcgaagcttttgatatctggggccaagggacaatggtcaccgtgtcctca

SEQ ID NO: 67 - DNA, 378 bp, Homo sapiens
caggtgcagctggtggcgtctgggggaggcttggtcaagcctggcgggtccctgagactctcctgtgcagcctctggattcaccttcagtgactactacatgacctggatccgccaggctccagggaaggggctggagtgggtctcgtatattagtagtagtggtacgaccatatactacgccgactctgtgaagggccgattcaccgtctccagggacaacgccaagaactcactgtttctgcaaatgaacagcctgagagccgaggacacggctctttattattgtgcgagagactcttattcgaagttggtggatatagaggccatcgaagcttttgatatctggggccaagggaccatggtcaccgtgtcctca

SEQ ID NO: 68 - DNA, 378 bp, Homo sapiens
caggtgcacctggtggagtctgggggaggcttggtcaagcctggacggtccctgagactctcctgtgcagcctctggattcaccttcagtgactattacatggcttggatccgccaagttccggggaaggggctggagtgggtttcattcattagtagtagtggtcgtaccatctactacgcagactctgtgaagggccgattcaccatctccagggacaacgccaaggactcactgtatcttcaaatgcacagcctgagagccgaggacacggctgtttattactgtgcgagagattcttattcgaagttggtggatatagaggccatcgaggcttttgatatctggggccgagggaccatggtcaccgtgtcctca

SEQ ID NO: 69 - DNA, 378 bp, Homo sapiens
caggtgcagctggtggaatctgggggaggcttggtcaagcctggagggtccctgagactctcctgtgcgccagctggattcaacttcaaagactactacatgacctggatccgccaggctccaggaaaggggctggagtgggtttccttcatcagtagtagtggtcagaccatatactacgcagactctgtgaagggccgattcaccatctccagggacaacgccaggaactcactgtatctgcaaatgaatagcctgagagccgaggacacggctgtttattactgtgcgagagactcttactcgaagttggtggatatagtggccatcgaagcttttgatctttggggccaagggacactggtcagcgtctcctca

SEQ ID NO: 70 - DNA, 378 bp, Homo sapiens
caggtgcagctggtggagtctgggggaggcctggtcaagcctggagggtccctgagactctcctgtgcagcctctggattcagcttcagtgcctactacatgagttggatccgccaggctccagggaaggggctggagtggatttcatacattagtagtagtggtaataccatatactacacagactctgtgaagggccgattcaccatcgccagggacaacgccaagaactcactttatctgcaaatgaacagcctgagagccgaggacacgggtctatattactgtgcgagagattcttattcgaagttggcggacatagaggccaccgaggcttttgatgtctggggccaagggacaatggtcgccgtctcttca

SEQ ID NO: 71 - DNA, 378 bp, Homo sapiens
caggtgcacctggtggagtctgggggaggcttggtcaagcctggagggtccctgagactctcctgtgcagcctctggattcaccttcagtgactattacatggcctggattcgccgcgctccggggaagggcctggagtggatttcattcattagtggcagcggccgcaccctctaccatgcagagtctgtgaagggccgattcaccgtctccagggacaacgccaaggactcactgtatcttcacatgcacagcctgagagacgcagacacggctgtttattactgtgcgagagattcttattcgaagttggtggaaatagaggccatcgaagcctttgatgtctggggccgagggacagtggtcaccgtctcctca

SEQ ID NO: 72 - DNA, 360 bp, Homo sapiens
cagctgcagttgcaggagtcgggcccaggactggtgaagccttcggagaccctgtccctcacctgctctgtctctggtgacgccatcagcggcagcaattattactggggctggatacgccagcccccagggaagggactgcagtggattgggagtatctatcacactgggagcaccttctacaacccgtcattcagcagtcgagtcaccttatccgtagacacgtccaagaaccagttctccctgaagctgatctctgtgaacgccgcagacacggctgtgtattattgtgcaagacggatcaggggttatagtgggacctacgactggggccagggaaccctggtcaccgtctcctca

SEQ ID NO: 73 - DNA, 387 bp, Homo sapiens
caggtgaagctggtggagtcggggggaggcgtggtccagcctgggaggtccctgagactctcatgtgcaggctctggattcgcctttgataactacgctatgcactgggtccgccaggctccaggcaaggggctggagtgggtggcagtcatatcacttgaaggaaggaataaatattacgcaggccccgcgaagggccggttctccatttccagagacaactccagaaacacagtgcatctgcaaatgaacagtctgagacctgaggacacggctgtgtatttctgtgcgagagatatgcgttactattatgatagtaatggtcactataggaaccgatatggcatggacgtctggggccaagggaccacggtcatcgtctcctca

SEQ ID NO: 74 - DNA, 357 bp, Homo sapiens
caggtgcagctggtgcagtctggagctgaggtgaagaagcctggggcctcagtgaaggtctcctgtaagacttctggttacacctttaatacttatgctatcagctgggtgcgccaggcccctggacaagggcttgagtgggtgggatggatcaacacttacagtggaagcacaaagtatgcacagaaggtccagggcagagtcaccatgaccacagacacatccacgagcaccgcctacatggagttgaggggcctgagatctgacgacacggccgtatattactgtgcgagagatggctacaattggggttttctcgacttctggggccagggatccctggtcaccgtctcctca

SEQ ID NO: 75 - DNA, 357 bp, Homo sapiens
caggtgcaggtggtgcagtctggagctgaggtgaagaagcctggggcctcagtgatggtctcctgcaagacttctggttacagatttaccatatatagtatcgcctggatgcgccaggccccgggacaagggcttgagtggatggggtcgatcaacacttacaatggcaatacaaagtatgcagagaagttccagggcagagtcaccatgagtagagacacatccacgagcacagcctacatggaggtgaggagcctgggatctgccgacacggccatgtattactgtgcgagagacgcagagaactggggattttttgacgactggggccaggggaccctggtcaccgtctcctca

SEQ ID NO: 76 - DNA, 375 bp, Homo sapiens
caggtgcagctggtggagtctgggggaggcgtggtccagcctggaaggtccctgagactctcctgtgcagcctctggattcaccttcagtaaccatggtctacactgggtccgccagcctccaggcaaggggctggagtgggtggcagttgtatcaaaagatggaaccaatgaacactacgcagactccgtgaggggccggttcaccatctccagagacaattccaagaacacgttgtatctgctaatgaagagcctcagacttgaggacacggctgtatattattgtgcgagagaagggtattgtggggatgatcgctgctactccggacagcctgactactggggccagggaatcctggtcaccgtctcctca

SEQ ID NO: 77 - protein, 128 aa, Homo sapiens
EVQLVQSGGGLVQPGGSLRVSCAASGFSFSDHDMDWVRQAPGKGFEWVGRSRNKDYSSTTEYAASVRGRFTISRHTSEDLLYLELNTVKTEDTAVYFCARGPHHSDRSGYYGGTFDIWGQGTMVTVSS

SEQ ID NO: 78 - protein, 122 aa, Homo sapiens
QVQLVESGAEVKKPGALVKVSCKASGYTFTNYAIHWVRQASGQRLEWMGWINAGRGNTKYSQKFQGRVTITRDTSASTAYMELSSLRSEDAAVYFCARDESTGDYYYYMDVWGKGTTVTVSS

SEQ ID NO: 79 - protein, 126 aa, Homo sapiens
QVQLVASGGGLVKPGGSLRLSCAASEFTFSDYYMTWIRQAPGKGLEWVSYISSSGTTIYYADSVKGRFTVSRDNAKNSLFLQMNSLRAEDTALYYCARDSYSKLVDIEAIEAFDIWGQGTMVTVSS

SEQ ID NO: 80 - protein, 126 aa, Homo sapiens
QVQLVASGGGLVKPGGSLRLSCAASGFTFSDYYMTWIRQAPGKGLEWVSYISSSGTTIYYADSVKGRFTVSRDNAKNSLFLQMNSLRAEDTALYYCARDSYSKLVDIEAIEAFDIWGQGTMVTVSS

SEQ ID NO: 81 - protein, 126 aa, Homo sapiens
QVHLVESGGGLVKPGRSLRLSCAASGFTFSDYYMAWIRQVPGKGLEWVSFISSSGRTIYYADSVKGRFTISRDNAKDSLYLQMHSLRAEDTAVYYCARDSYSKLVDIEAIEAFDIWGRGTMVTVSS

SEQ ID NO: 82 - protein, 126 aa, Homo sapiens
QVQLVESGGGLVKPGGSLRLSCAPAGFNFKDYYMTWIRQAPGKGLEWVSFISSSGQTIYYADSVKGRFTISRDNARNSLYLQMNSLRAEDTAVYYCARDSYSKLVDIVAIEAFDLWGQGTLVSVSS

SEQ ID NO: 83 - protein, 126 aa, Homo sapiens
QVQLVESGGGLVKPGGSLRLSCAASGFSFSAYYMSWIRQAPGKGLEWISYISSSGNTIYYTDSVKGRFTIARDNAKNSLYLQMNSLRAEDTGLYYCARDSYSKLADIEATEAFDVWGQGTMVAVSS

SEQ ID NO: 84 - protein, 126 aa, Homo sapiens
QVHLVESGGGLVKPGGSLRLSCAASGFTFSDYYMAWIRRAPGKGLEWISFISGSGRTLYHAESVKGRFTVSRDNAKDSLYLHMHSLRDADTAVYYCARDSYSKLVEIEAIEAFDVWGRGTVVTVSS

SEQ ID NO: 85 - protein, 120 aa, Homo sapiens
QLQLQESGPGLVKPSETLSLTCSVSGDAISGSNYYWGWIRQPPGKGLQWIGSIYHTGSTFYNPSFSSRVTLSVDTSKNQFSLKLISVNAADTAVYYCARRIRGYSGTYDWGQGTLVTVSS

SEQ ID NO: 86 - protein, 129 aa, Homo sapiens
QVKLVESGGGVVQPGRSLRLSCAGSGFAFDNYAMHWVRQAPGKGLEWVAVISLEGRNKYYAGPAKGRFSISRDNSRNTVHLQMNSLRPEDTAVYFCARDMRYYYDSNGHYRNRYGMDVWGQGTTVIVSS

SEQ ID NO: 87 - protein, 119 aa, Homo sapiens
QVQLVQSGAEVKKPGASVKVSCKTSGYTFNTYAISWVRQAPGQGLEWVGWINTYSGSTKYAQKVQGRVTMTTDTSTSTAYMELRGLRSDDTAVYYCARDGYNWGFLDFWGQGSLVTVSS

SEQ ID NO: 88 - protein, 119 aa, Homo sapiens
QVQVVQSGAEVKKPGASVMVSCKTSGYRFTIYSIAWMRQAPGQGLEWMGSINTYNGNTKYAEKFQGRVTMSRDTSTSTAYMEVRSLGSADTAMYYCARDAENWGFFDDWGQGTLVTVSS

SEQ ID NO: 89 - protein, 125 aa, Homo sapiens
QVQLVESGGGVVQPGRSLRLSCAASGFTFSNHGLHWVRQPPGKGLEWVAVVSKDGTNEHYADSVRGRFTISRDNSKNTLYLLMKSLRLEDTAVYYCAREGYCGDDRCYSGQPDYWGQGILVTVSS

SEQ ID NO: 90 - DNA, 321 bp, Homo sapiens
gacatccagatgacccagtctccatcttccgtgtctgcatctgtaggcgacagagtcatcatcacttgtcgggcgagtcagggtattagcagctggttagcctggtatcagcagaaaccagggagagccccgaggctcctgatctatgatgcctccactttggaaagtggggtcccatcaaggttcagcggcagaggatctgggacagaattcactctcaccatcaacagcctgcagcctgaagattttgcaacttactattgtcaacagggtaacatgttcccgctcactttcggcggagggaccaaggtggaaatcaaa

SEQ ID NO: 91 - DNA, 318 bp, Homo sapiens
tcctatgagctgactcagccaccctcagtgtccgtgtccccaggacagacagccagcatcacctgctctggagatagattggacgataaatatgcttcctggtatcagcagaaggcaggccagtcccctgtcctggtcatctatcaagataacaagaggccctcagggatccctgagcgattctctggctccaactctgggaacactgccactctgaccatcagcgggacccaggctatggatgaggctgactattattgtcaggcgtgggacagcgacacgtatgtcttcggaactgggaccaaggtcaccgtccta

SEQ ID NO: 92 - DNA, 324 bp, Homo sapiens
tcctatgagctgactcagccaccctcagtgtcagtgggcccgggaaggacggccaggattacctgtggggcaaacaacattggaagtaaaagtgtgcactggtaccaacagaggcctggccaggcccctgtcctggtcatctcttttgataccgaccggccctcagggatccctgagcgattctctggctccaactctgggaacacggccaccctgaccatcagcagggtcgaagccggggatgaggccgactatttctgtcaggtgtgggatcgtactagtgatcatgtggtgttcggcggagggaccaagctgaccgtccta

SEQ ID NO: 93 - DNA, 324 bp, Homo sapiens
tcctatgagctggctcagccaccctcagtgtcagtggccccaggaaagacggccacgattgcctgtgggggagacaatattggaggtaaaagtgtgcactggtaccttcagaaggcaggccaggcccctgtattggtcatttcttatgacagcgaccggccctcagggatccctgagcgattctctggctccaactctgggaacacggccaccctgaccatcagcagggtcgaagccggtgatgaggccgactatttctgtcaggtgtgggatcgtcatggtgatcatgtggtcttcggcggagggaccaagctgaccgtccta

SEQ ID NO: 94 - DNA, 324 bp, Homo sapiens
tcctatgagctgactcaaccaccctcagtgtcagtggccccaggaaaaatggccaggattacctgtggcggagacaacattggaagtaaaagtgtgcactggtaccagcagaggccaggccaggcccctgtcctggtcatccgttttgataccgaccggccctcacggatccctgagcgattctctggctccaactcagggaacacggccaccctggccatcagcagggtcgaagccggggatgaggccgactattactgtcaggtgtgggattctagtagtgctcgtttggtgttcggcggagggaccaagctgaccgtccta

SEQ ID NO: 95 - DNA, 324 bp, Homo sapiens
tcctatgagctgactcagcctccctcagtgtcagtggccccaggaaagacggccaggattacttgtgggggaaacaacattggaagtaagagtgtgcactggtaccagcagaagccaggccaggcccctgtcatggtcatctattatgatagcgaccggccctcagggatccctgagcgattctctggctccaactctgggaacacggccactctgaccatcagcagggtcgaagccggggatgaggccgactattactgtcaggtgtgggatagtggtagtgatcgtgtggtattcggcggagggaccaagctgaccgtccta

SEQ ID NO: 96 - DNA, 324 bp, Homo sapiens
tcctatgagctggctcagccaccctcagtgtcagtggccccaggaaagccggccaggattgcctgtgggggagacaacattggaggtaaaagtgtgcactggtaccttcagaaggcaggccaggcccctgtcctggtcatgtcttatgacagcgaccggccctcagggatccctgagcgattctctggctccaactctggcaacacggccaccctgaccatcagcagggtcgaagccggtgatgaaggcgactatttctgtcaggtgtgggatcgtcaaactgatcatgtggtcttcggcggagggaccaagctgaccgtccta

SEQ ID NO: 97 - DNA, 309 bp, Homo sapiens
gacatccagttgacccagtctccgtccttcctgtctgcatctgtaggcgacagagtcaccatcacttgccgggccagtcaggacataagcagttatgtagcctggtatcagcaaaaaccagggaatgcccctaagctcctgatctcttctgcatccactttgccaagtggggtcccgtcaaggttcagcggcagtagatctgggacagacttcactctcacaatcagcagcctgcagcctgaagattttgcaacttattactgtcaacaacttaataatttcggccctgggactacagtggatatcaaa

SEQ ID NO: 98 - DNA, 318 bp, Homo sapiens
gacatccagatgacccaatctccatcctccctgtctgcgtctgtaggagacagcgtcaccatcacttgccaggcgagtcaggacattaatcagtttgtaagttggtatcaacagaaaccagggaaaccccctaaactcctgatctacgatgcttccaatttggagtcaggcgtcccatcaaggttcagtggaagtggatctgggacacattttactttcaccatcagcagcctgcagcccgacgatattgcgacatattactgtcagcaatatgaaaatctattcactttcggccctgggaccaaagtggatatcaaa

SEQ ID NO: 99 - DNA, 321 bp, Homo sapiens
gacatccagatgacccagtctccatcctccctgtctgcatctgtaggagacagagtcaccatcacttgccgggcgagtcagggcattagcaattatttagcctggtatcagcaaaaaccggggaaacttcctaagctcctgatctatgctgcatccacgttgcaatcaggggtcccatctcggttcagtggcagtggatctgggacagatttcactctcaccatcagcagcctgcagcctgaagatgttgcaagttattactgtcaaaagtataacagtgcccctctcactttcggccctgggaccaaagtggatatcaaa

SEQ ID NO: 100 - DNA, 321 bp, Homo sapiens
gaaattgtgttgacgcagtctccaggcactgtgtctttgtctcccggggaaagagtcaccctctcctgcagggccagtcagagtgtcggcagacacttagcctggtaccagcagaaacctggccagcctcccaggctcctcatctatggtgcatctaccagggccactggcgtcccagacaggttcagtggcagtgggtctgagacagagttcactctcgccatcagcagcctgcagtctgaagattttgcactttattactgtcaacaatataatacctggccgtacacttttggccaggggaccaagctggagatcaaa

SEQ ID NO: 101 - DNA, 324 bp, Homo sapiens
gaaattgtgttgacacagtttccagccaccctgtctttgtctccaggagaaagagccaccctctcctgcagggccagtcagagtgttggcaggtacttggcctggtaccaacagaaacctggccaggctcccaggctcctcatctatgattcatccaacagggccactggcgtcccagccaggttcagtggcagtgggtctgggacagacttcactctctccatcagcagcctggagcctgaagattttgcagtgtatttctgtcaacagcgtagccactggcctccgctcactttcggcggagggaccaaggtggaaatcaaa

SEQ ID NO: 102 - protein, 107 aa, Homo sapiens
DIQMTQSPSSVSASVGDRVIITCRASQGISSWLAWYQQKPGRAPRLLIYDASTLESGVPSRFSGRGSGTEFTLTINSLQPEDFATYYCQQGNMFPLTFGGGTKVEIK

SEQ ID NO: 103 - protein, 106 aa, Homo sapiens
SYELTQPPSVSVSPGQTASITCSGDRLDDKYASWYQQKAGQSPVLVIYQDNKRPSGIPERFSGSNSGNTATLTISGTQAMDEADYYCQAWDSDTYVFGTGTKVTVL

SEQ ID NO: 104 - protein, 108 aa, Homo sapiens
SYELTQPPSVSVGPGRTARITCGANNIGSKSVHWYQQRPGQAPVLVISFDTDRPSGIPERFSGSNSGNTATLTISRVEAGDEADYFCQVWDRTSDHVVFGGGTKLTVL

SEQ ID NO: 105 - protein, 108 aa, Homo sapiens
SYELAQPPSVSVAPGKTATIACGGDNIGGKSVHWYLQKAGQAPVLVISYDSDRPSGIPERFSGSNSGNTATLTISRVEAGDEADYFCQVWDRHGDHVVFGGGTKLTVL

SEQ ID NO: 106 - protein, 108 aa, Homo sapiens
SYELTQPPSVSVAPGKMARITCGGDNIGSKSVHWYQQRPGQAPVLVIRFDTDRPSRIPERFSGSNSGNTATLAISRVEAGDEADYYCQVWDSSSARLVFGGGTKLTVL

SEQ ID NO: 107 - protein, 108 aa, Homo sapiens
SYELTQPPSVSVAPGKTARITCGGNNIGSKSVHWYQQKPGQAPVMVIYYDSDRPSGIPERFSGSNSGNTATLTISRVEAGDEADYYCQVWDSGSDRVVFGGGTKLTVL

SEQ ID NO: 108 - protein, 108 aa, Homo sapiens
SYELAQPPSVSVAPGKPARIACGGDNIGGKSVHWYLQKAGQAPVLVMSYDSDRPSGIPERFSGSNSGNTATLTISRVEAGDEGDYFCQVWDRQTDHVVFGGGTKLTVL

SEQ ID NO: 109 - protein, 103 aa, Homo sapiens
DIQLTQSPSFLSASVGDRVTITCRASQDISSYVAWYQQKPGNAPKLLISSASTLPSGVPSRFSGSRSGTDFTLTISSLQPEDFATYYCQQLNNFGPGTTVDIK

SEQ ID NO: 110 - protein, 106 aa, Homo sapiens
DIQMTQSPSSLSASVGDSVTITCQASQDINQFVSWYQQKPGKPPKLLIYDASNLESGVPSRFSGSGSGTHFTFTISSLQPDDIATYYCQQYENLFTFGPGTKVDIK

SEQ ID NO: 111 - protein, 107 aa, Homo sapiens
DIQMTQSPSSLSASVGDRVTITCRASQGISNYLAWYQQKPGKLPKLLIYAASTLQSGVPSRFSGSGSGTDFTLTISSLQPEDVASYYCQKYNSAPLTFGPGTKVDIK

SEQ ID NO: 112 - protein, 107 aa, Homo sapiens
EIVLTQSPGTVSLSPGERVTLSCRASQSVGRHLAWYQQKPGQPPRLLIYGASTRATGVPDRFSGSGSETEFTLAISSLQSEDFALYYCQQYNTWPYTFGQGTKLEIK

SEQ ID NO: 113 - protein, 108 aa, Homo sapiens
EIVLTQFPATLSLSPGERATLSCRASQSVGRYLAWYQQKPGQAPRLLIYDSSNRATGVPARFSGSGSGTDFTLSISSLEPEDFAVYFCQQRSHWPPLTFGGGTKVEIK

SEQ ID NO: 114 - DNA, 384 bp, Artificial Sequence
  GERMLINED 2-18 IgG1 HEAVY CHAIN
gaggtgcagctggtggagtctggaggaggactggtgcagccaggaggctccctgaggctgtcttgcgccgccagcggcttctccttttctgaccacgatatggactgggtgcgccaggcacctggcaagggcctggagtgggtgggccggagcagaaacaaggattacagctccaccacagagtatgcagcctccgtgaggggccgcttcaccatctctcgggacgatagcaagaactccctgtacctgcagatgaacagcctgaagaccgaggacacagccgtgtactattgtgccagaggcccccaccactctgatagaagcggctactatggcggcacatttgacatctggggccagggcacaatggtgacagtgtctagc

SEQ ID NO: 115 - protein, 128 aa, Artificial Sequence
  GERMLINED 2-18 IgG1 HEAVY CHAIN
EVQLVESGGGLVQPGGSLRLSCAASGFSFSDHDMDWVRQAPGKGLEWVGRSRNKDYSSTTEYAASVRGRFTISRDDSKNSLYLQMNSLKTEDTAVYYCARGPHHSDRSGYYGGTFDIWGQGTMVTVSS

SEQ ID NO: 116 - DNA, 321 bp, Artificial Sequence
  GERMLINED 2-18 IgG1 LIGHT CHAIN
gacatccagatgacacagtctcctagctccgtgagcgcctccgtgggcgatagggtgaccatcacatgcagagcctcccagggcatctctagctggctggcctggtatcagcagaagcccggcaaggcccctaagctgctgatctatgacgcctctaccctggagagcggcgtgccctcccggttctctggcagcggctccggcacagactttaccctgacaatctcctctctgcagccagaggatttcgccacctactattgtcagcagggcaacatgttccccctgacctttggcggcggcacaaaggtggagatcaag

SEQ ID NO: 117 - protein, 107 aa, Artificial Sequence
  GERMLINED 2-18 IgG1 LIGHT CHAIN
DIQMTQSPSSVSASVGDRVTITCRASQGISSWLAWYQQKPGKAPKLLIYDASTLESGVPSRFSGSGSGTDFTLTISSLQPEDFATYYCQQGNMFPLTFGGGTKVEIK

SEQ ID NO: 118 - DNA, 378 bp, Artificial Sequence
  GERMLINED 1-85 IgG1 HEAVY CHAIN
caggtgcagctggtggagtccggaggaggactggtgaagccaggaggctccctgaggctgtcttgcgccgccagcggcttcacctttagcgactactatatggcctggatcagacaggcacctggcaagggcctggagtgggtgtccttcatcagctcctctggcagaaccatctactatgccgactctgtgaagggccggtttacaatctccagagataacgccaagaacagcctgtacctgcagatgaacagcctgagggccgaggacacagccgtgtactattgtgcccgcgactcttatagcaagctggtggatatcgaggccatcgaggccttcgatatctggggcagaggcacaatggtgaccgtgagcagc

SEQ ID NO: 119 - protein, 126 aa, Artificial Sequence
  GERMLINED 1-85 IgG1 HEAVY CHAIN
QVQLVESGGGLVKPGGSLRLSCAASGFTFSDYYMAWIRQAPGKGLEWVSFISSSGRTIYYADSVKGRFTISRDNAKNSLYLQMNSLRAEDTAVYYCARDSYSKLVDIEAIEAFDIWGRGTMVTVSS

SEQ ID NO: 120 - DNA, 324 bp, Artificial Sequence
  GERMLINED 1-85 IgG1 LIGHT CHAIN
agctacgtgctgacacagccacctagcgtgtccgtggcaccaggcaagacagcaaggatcacctgcggcggcgacaacatcggctctaagagcgtgcactggtatcagcagaagccaggacaggcacccgtgctggtcatctactatgactccgatcggccttctggcatcccagagagattctccggctctaacagcggcaataccgccacactgaccatctccagggtggaggcaggcgacgaggcagattacttctgtcaagtgtgggaccgccacggcgatcacgtggtgtttggcggcggcacaaagctgaccgtgctg

SEQ ID NO: 121 - protein, 108 aa, Artificial Sequence
  GERMLINED 1-85 IgG1 LIGHT CHAIN
SYVLTQPPSVSVAPGKTARITCGGDNIGSKSVHWYQQKPGQAPVLVIYYDSDRPSGIPERFSGSNSGNTATLTISRVEAGDEADYFCQVWDRHGDHVVFGGGTKLTVL

SEQ ID NO: 122 - DNA, 375 bp, Artificial Sequence
  GERMLINED 3-25 HEAVY CHAIN
caggtgcagctggtggagagcggaggaggagtggtgcagccaggcaggtctctgaggctgagctgcgccgcctccggcttcaccttttccaaccacggcctgcactgggtgcggcaggcacctggcaagggcctggagtgggtggcagtggtgtccaaggacggcacaaatgagcactacgccgattctgtgcggggcagattcaccatctctagggacaacagcaagaatacactgtatctgcagatgaactctctgcgcgccgaggataccgccgtgtactattgtgcccgggagggctactgcggcgacgatagatgttacagcggacagccagactattggggacagggcaccctggtgaccgtgagcagc

SEQ ID NO: 123 - protein, 125 aa, Artificial Sequence
  GERMLINED 3-25 HEAVY CHAIN
QVQLVESGGGVVQPGRSLRLSCAASGFTFSNHGLHWVRQAPGKGLEWVAVVSKDGTNEHYADSVRGRFTISRDNSKNTLYLQMNSLRAEDTAVYYCAREGYCGDDRCYSGQPDYWGQGTLVTVSS

SEQ ID NO: 124 - DNA, 324 bp, Artificial Sequence
  GERMLINED 3-25 LIGHT CHAIN
gagatcgtgctgacccagtctcctgccacactgtccctgtctccaggagagagggccaccctgagctgcagagccagccagtccgtgggcagatacctggcctggtatcagcagaagccaggacaggcaccaaggctgctgatctacgacagctccaacagggcaaccggcgtgcccgcacgcttctctggcagcggctccggcacagactttaccctgacaatctctagcctggagcctgaggatttcgccgtgtactattgtcagcagcggtcccactggccacctctgacctttggcggaggcacaaaggtggagatcaag

SEQ ID NO: 125 - protein, 108 aa, Artificial Sequence
  GERMLINED 3-25 LIGHT CHAIN
EIVLTQSPATLSLSPGERATLSCRASQSVGRYLAWYQQKPGQAPRLLIYDSSNRATGVPARFSGSGSGTDFTLTISSLEPEDFAVYYCQQRSHWPPLTFGGGTKVEIK

SEQ ID NO: 126 - DNA, 1374 bp, Artificial Sequence
  GERMLINED 2-18 IgG1 HEAVY CHAIN
gaggtgcagctggtggagtctggaggaggactggtgcagccaggaggctccctgaggctgtcttgcgccgccagcggcttctccttttctgaccacgatatggactgggtgcgccaggcacctggcaagggcctggagtgggtgggccggagcagaaacaaggattacagctccaccacagagtatgcagcctccgtgaggggccgcttcaccatctctcgggacgatagcaagaactccctgtacctgcagatgaacagcctgaagaccgaggacacagccgtgtactattgtgccagaggcccccaccactctgatagaagcggctactatggcggcacatttgacatctggggccagggcacaatggtgacagtgtctagcgcatccaccaagggcccatctgtcttccccctggccccatcctccaagagcacctctggcggcacagctgccctgggctgcctggtgaaggactacttccctgagcctgtgacagtgtcctggaactctggcgccctgaccagcggcgtgcacaccttccctgctgtgctccagtcctctggcctgtactccctgagcagcgtggtgacagtgccatccagcagcctgggcacccagacctacatctgcaatgtgaaccacaagcccagcaacaccaaggtggacaagcgggtggagcccaagtcctgtgacaagacccacacctgccccccatgccccgcccctgagctgctgggcggcccatctgtcttcctgttcccccccaagcccaaggacaccctgatgatctcccggacccccgaggtgacctgtgtggtggtggatgtgagccatgaggaccccgaggtgaagttcaactggtatgtggatggcgtggaggtgcacaacgccaagaccaagccccgggaggagcagtacaacagcacctaccgggtggtgagcgtgctgacagtgctgcatcaggactggctgaatggcaaggagtacaagtgcaaggtgtccaacaaggccctgcctgcccccattgagaagaccatctccaaggccaagggccagccccgggagccccaggtctacaccctgcccccctcccgggaggagatgaccaagaaccaggtgagcctgacctgcctggtgaagggcttctaccccagcgacattgctgtggagtgggagagcaacggccagcctgagaacaactacaagaccaccccccctgtgctggactctgatggctccttcttcctgtacagcaagctgacagtggacaagagccggtggcagcagggcaatgtcttctcctgctctgtgatgcatgaggccctgcacaaccactacacccagaagagcctgtccctgtcccccggcaag

SEQ ID NO: 127 - protein, 458 aa, Artificial Sequence
  GERMLINED 2-18 IgG1 HEAVY CHAIN
EVQLVESGGGLVQPGGSLRLSCAASGFSFSDHDMDWVRQAPGKGLEWVGRSRNKDYSSTTEYAASVRGRFTISRDDSKNSLYLQMNSLKTEDTAVYYCARGPHHSDRSGYYGGTFDIWGQGTMVTVSSASTKGPSVFPLAPSSKSTSGGTAALGCLVKDYFPEPVTVSWNSGALTSGVHTFPAVLQSSGLYSLSSVVTVPSSSLGTQTYICNVNHKPSNTKVDKRVEPKSCDKTHTCPPCPAPELLGGPSVFLFPPKPKDTLMISRTPEVTCVVVDVSHEDPEVKFNWYVDGVEVHNAKTKPREEQYNSTYRVVSVLTVLHQDWLNGKEYKCKVSNKALPAPIEKTISKAKGQPREPQVYTLPPSREEMTKNQVSLTCLVKGFYPSDIAVEWESNGQPENNYKTTPPVLDSDGSFFLYSKLTVDKSRWQQGNVFSCSVMHEALHNHYTQKSLSLSPGK

SEQ ID NO: 128 - DNA, 642 bp, Artificial Sequence
  GERMLINED 2-18 IgG1 LIGHT CHAIN
gacatccagatgacacagtctcctagctccgtgagcgcctccgtgggcgatagggtgaccatcacatgcagagcctcccagggcatctctagctggctggcctggtatcagcagaagcccggcaaggcccctaagctgctgatctatgacgcctctaccctggagagcggcgtgccctcccggttctctggcagcggctccggcacagactttaccctgacaatctcctctctgcagccagaggatttcgccacctactattgtcagcagggcaacatgttccccctgacctttggcggcggcacaaaggtggagatcaagcgtacggtggctgcaccatctgtcttcatcttcccgccatctgatgagcagttgaaatctggaactgcctctgttgtgtgcctgctgaataacttctatcccagagaggccaaagtacagtggaaggtggataacgccctccaatcgggtaactcccaggagagtgtcacagagcaggacagcaaggacagcacctacagcctcagcagcaccctgacgctgagcaaagcagactacgagaaacacaaagtctacgcctgcgaagtcacccatcagggcctgagctcgcccgtcacaaagagcttcaacaggggagagtgt

SEQ ID NO: 129 - protein, 214 aa, Artificial Sequence
  GERMLINED 2-18 IgG1 LIGHT CHAIN
DIQMTQSPSSVSASVGDRVTITCRASQGISSWLAWYQQKPGKAPKLLIYDASTLESGVPSRFSGSGSGTDFTLTISSLQPEDFATYYCQQGNMFPLTFGGGTKVEIKRTVAAPSVFIFPPSDEQLKSGTASVVCLLNNFYPREAKVQWKVDNALQSGNSQESVTEQDSKDSTYSLSSTLTLSKADYEKHKVYACEVTHQGLSSPVTKSFNRGEC

SEQ ID NO: 130 - DNA, 1434 bp, Artificial Sequence
  GERMLINED 2-18 IgG1 HEAVY CHAIN + YTE
atggagtggagctgggtgtttctgttcttcctcagcgtgaccaccggcgtgcattccgaggtgcagctggtggagtccggaggaggactcgtgcagcccggaggttctctgaggctcagctgtgctgcctccggattctccttcagcgaccacgacatggattgggtgcggcaggctcccggaaaaggcctggagtgggtcggcaggagcaggaacaaggactattccagcaccaccgaatacgccgccagcgtgaggggcaggttcaccatctccagggatgacagcaagaactccctgtacctgcagatgaacagcctgaagaccgaagacaccgccgtgtactattgcgcccggggccctcaccattccgaccggagcggctattacggcggcaccttcgacatttggggccagggaacaatggtcaccgtgtccagcgctagcaccaagggccctagcgtgttccccctggctcctagctccaagagcaccagcggaggcacagccgctctgggatgcctggtcaaagactacttccccgagcccgtcacagtcagctggaactccggagccctgacctccggcgtccataccttccccgctgtgctgcagagctccggcctgtactccctgagctccgtggtcacagtgcctagctccagcctcggaacccagacatacatctgcaacgtgaaccacaagccctccaacaccaaggtcgacaagaaggtggagcctaagtcctgcgacaaaacccacacctgccctccttgccctgctcctgaactgctgggcggcccttccgtgttcctgttcccccctaaacctaaggacaccctgtacatcacccgggagcccgaggtgacatgcgtggtggtggacgtgtcccacgaggaccccgaggtgaagttcaactggtatgtcgatggcgtggaggtccacaacgccaagaccaaacccagggaagagcagtacaactccacctaccgggtggtcagcgtgctgaccgtgctgcaccaggactggctgaatggcaaggagtacaagtgcaaggtcagcaataaagccctgcccgcccctatcgagaagacaatctccaaggccaagggacagcccagggaaccccaggtgtataccctgcccccctcccgggatgaactgaccaaaaaccaggtcagcctgacctgtctggtcaaaggcttctacccctccgacatcgctgtggaatgggagagcaatggccagcctgagaacaactataagaccacccctcccgtgctcgacagcgatggctccttctttctctacagcaagctgaccgtggataagtcccggtggcaacagggcaacgtgttcagctgctccgtcatgcatgaggccctgcacaatcactacacccagaagagcctgtccctgtcccccggcaagtga

SEQ ID NO: 131 - protein, 477 aa, Artificial Sequence
  GERMLINED 2-18 IgG1 HEAVY CHAIN + YTE
MEWSWVFLFFLSVTTGVHSEVQLVESGGGLVQPGGSLRLSCAASGFSFSDHDMDWVRQAPGKGLEWVGRSRNKDYSSTTEYAASVRGRFTISRDDSKNSLYLQMNSLKTEDTAVYYCARGPHHSDRSGYYGGTFDIWGQGTMVTVSSASTKGPSVFPLAPSSKSTSGGTAALGCLVKDYFPEPVTVSWNSGALTSGVHTFPAVLQSSGLYSLSSVVTVPSSSLGTQTYICNVNHKPSNTKVDKKVEPKSCDKTHTCPPCPAPELLGGPSVFLFPPKPKDTLYITREPEVTCVVVDVSHEDPEVKFNWYVDGVEVHNAKTKPREEQYNSTYRVVSVLTVLHQDWLNGKEYKCKVSNKALPAPIEKTISKAKGQPREPQVYTLPPSRDELTKNQVSLTCLVKGFYPSDIAVEWESNGQPENNYKTTPPVLDSDGSFFLYSKLTVDKSRWQQGNVFSCSVMHEALHNHYTQKSLSLSPGK

SEQ ID NO: 132 - DNA, 705 bp, Artificial Sequence
  GERMLINED 2-18 IgG1 LIGHT CHAIN + YTE
atgagcgtgcccacacaggtgctcggcctgctgctgctgtggctgaccgacgccaggtgcgacatccagatgacccagtccccttcctccgtgtccgcttccgtgggcgatagggtgacaatcacctgcagggccagccagggcatctccagctggctggcctggtaccagcagaagcccggcaaggcccccaagctgctgatctacgacgccagcacactggagagcggcgtgccttcccggttcagcggttctggcagcggaacagacttcaccctgaccatttcctccctgcagcccgaggacttcgccacctactactgccagcagggcaacatgttccctctgaccttcggaggcggcacaaaggtggagatcaagcggaccgtcgccgctccctccgtgttcatcttccccccctccgatgagcagctcaagtccggcaccgctagcgtggtgtgcctgctgaacaacttctacccccgggaggccaaggtgcagtggaaggtcgacaacgccctgcagtccggcaacagccaggagagcgtgaccgagcaggactccaaggactccacctactccctctcctccaccctgaccctgtccaaggccgactacgagaagcacaaagtgtacgcctgcgaagtgacccaccagggcctgagctcccccgtgacaaagtccttcaacaggggcgagtgttga

SEQ ID NO: 133 - protein, 234 aa, Artificial Sequence
  GERMLINED 2-18 IgG1 LIGHT CHAIN + YTE
MSVPTQVLGLLLLWLTDARCDIQMTQSPSSVSASVGDRVTITCRASQGISSWLAWYQQKPGKAPKLLIYDASTLESGVPSRFSGSGSGTDFTLTISSLQPEDFATYYCQQGNMFPLTFGGGTKVEIKRTVAAPSVFIFPPSDEQLKSGTASVVCLLNNFYPREAKVQWKVDNALQSGNSQESVTEQDSKDSTYSLSSTLTLSKADYEKHKVYACEVTHQGLSSPVTKSFNRGEC

SEQ ID NO: 134 - DNA, 1368 bp, Artificial Sequence
  GERMLINED 1-85 IgG1 HEAVY CHAIN
caggtgcagctggtggagtccggaggaggactggtgaagccaggaggctccctgaggctgtcttgcgccgccagcggcttcacctttagcgactactatatggcctggatcagacaggcacctggcaagggcctggagtgggtgtccttcatcagctcctctggcagaaccatctactatgccgactctgtgaagggccggtttacaatctccagagataacgccaagaacagcctgtacctgcagatgaacagcctgagggccgaggacacagccgtgtactattgtgcccgcgactcttatagcaagctggtggatatcgaggccatcgaggccttcgatatctggggcagaggcacaatggtgaccgtgagcagcgcatccaccaagggcccatctgtcttccccctggccccatcctccaagagcacctctggcggcacagctgccctgggctgcctggtgaaggactacttccctgagcctgtgacagtgtcctggaactctggcgccctgaccagcggcgtgcacaccttccctgctgtgctccagtcctctggcctgtactccctgagcagcgtggtgacagtgccatccagcagcctgggcacccagacctacatctgcaatgtgaaccacaagcccagcaacaccaaggtggacaagcgggtggagcccaagtcctgtgacaagacccacacctgccccccatgccccgcccctgagctgctgggcggcccatctgtcttcctgttcccccccaagcccaaggacaccctgatgatctcccggacccccgaggtgacctgtgtggtggtggatgtgagccatgaggaccccgaggtgaagttcaactggtatgtggatggcgtggaggtgcacaacgccaagaccaagccccgggaggagcagtacaacagcacctaccgggtggtgagcgtgctgacagtgctgcatcaggactggctgaatggcaaggagtacaagtgcaaggtgtccaacaaggccctgcctgcccccattgagaagaccatctccaaggccaagggccagccccgggagccccaggtctacaccctgcccccctcccgggaggagatgaccaagaaccaggtgagcctgacctgcctggtgaagggcttctaccccagcgacattgctgtggagtgggagagcaacggccagcctgagaacaactacaagaccaccccccctgtgctggactctgatggctccttcttcctgtacagcaagctgacagtggacaagagccggtggcagcagggcaatgtcttctcctgctctgtgatgcatgaggccctgcacaaccactacacccagaagagcctgtccctgtcccccggcaag

SEQ ID NO: 135 - protein, 456 aa, Artificial Sequence
  GERMLINED 1-85 IgG1 HEAVY CHAIN
QVQLVESGGGLVKPGGSLRLSCAASGFTFSDYYMAWIRQAPGKGLEWVSFISSSGRTIYYADSVKGRFTISRDNAKNSLYLQMNSLRAEDTAVYYCARDSYSKLVDIEAIEAFDIWGRGTMVTVSSASTKGPSVFPLAPSSKSTSGGTAALGCLVKDYFPEPVTVSWNSGALTSGVHTFPAVLQSSGLYSLSSVVTVPSSSLGTQTYICNVNHKPSNTKVDKRVEPKSCDKTHTCPPCPAPELLGGPSVFLFPPKPKDTLMISRTPEVTCVVVDVSHEDPEVKFNWYVDGVEVHNAKTKPREEQYNSTYRVVSVLTVLHQDWLNGKEYKCKVSNKALPAPIEKTISKAKGQPREPQVYTLPPSREEMTKNQVSLTCLVKGFYPSDIAVEWESNGQPENNYKTTPPVLDSDGSFFLYSKLTVDKSRWQQGNVFSCSVMHEALHNHYTQKSLSLSPGK

SEQ ID NO: 136 - DNA, 639 bp, Artificial Sequence
  GERMLINED 1-85 IgG1 LIGHT CHAIN
agctacgtgctgacacagccacctagcgtgtccgtggcaccaggcaagacagcaaggatcacctgcggcggcgacaacatcggctctaagagcgtgcactggtatcagcagaagccaggacaggcacccgtgctggtcatctactatgactccgatcggccttctggcatcccagagagattctccggctctaacagcggcaataccgccacactgaccatctccagggtggaggcaggcgacgaggcagattacttctgtcaagtgtgggaccgccacggcgatcacgtggtgtttggcggcggcacaaagctgaccgtgctgcagcccaaggccaaccccaccgtgaccctgttccccccatcttctgaggagctgcaagccaacaaggccaccctggtgtgcctgatctctgacttctaccctggcgctgtgacagtggcctggaaggctgatggctctcctgtgaaggctggcgtggagaccaccaagccatctaagcagtctaacaacaagtatgctgcctcttcttacctgtctctgacccctgagcagtggaagagccaccggtcttactcttgccaggtgacccatgagggctctacagtggagaagacagtggcccccacagagtgctct

SEQ ID NO: 137 - protein, 213 aa, Artificial Sequence
  GERMLINED 1-85 IgG1 LIGHT CHAIN
SYVLTQPPSVSVAPGKTARITCGGDNIGSKSVHWYQQKPGQAPVLVIYYDSDRPSGIPERFSGSNSGNTATLTISRVEAGDEADYFCQVWDRHGDHVVFGGGTKLTVLQPKANPTVTLFPPSSEELQANKATLVCLISDFYPGAVTVAWKADGSPVKAGVETTKPSKQSNNKYAASSYLSLTPEQWKSHRSYSCQVTHEGSTVEKTVAPTECS

SEQ ID NO: 138 - DNA, 1428 bp, Artificial Sequence
  GERMLINED 1-85 IgG1 HEAVY CHAIN + YTE
atggaatggtcctgggtgttcctgttctttctgagcgtcaccaccggcgtgcacagcgaggtgcaactggtggagagcggcggaggcctggtgaaacctggcggttctctgaggctgtcctgtgctgccagcggcttcaccttctccgactattacatggcctggattcggcaggctcctggcaagggcctggaatgggtgtccttcatctccagcagcggccggacaatctattatgccgactccgtgaagggccggtttaccatctccagggataacgccaagaactccctgtacctgcagatgaactctctgagggctgaagacacagctgtgtattactgcgctcgggacagctacagcaagctggtggatatcgaggccatcgaagccttcgatatttggggcaggggaaccatggtgaccgtgagctccgcttccaccaagggacccagcgtgttccctctggctcctagctccaagtccaccagcggaggcaccgctgctctgggatgtctggtgaaagactactttcccgagcctgtcacagtgtcctggaacagcggagccctgaccagcggagtccacaccttccccgctgtgctgcagtcctccggcctgtacagcctgagcagcgtggtgaccgtgccttccagctccctcggcacccagacctacatctgcaatgtgaatcacaagcccagcaacaccaaggtggataagaaggtcgagcctaagagctgcgacaagacccacacatgccctccttgtcctgctcctgagctgctgggaggccctagcgtcttcctcttccctcccaaacccaaggataccctctacatcacccgggagcccgaagtgacctgcgtggtggtggacgtgtcccacgaagatcctgaagtcaagttcaactggtacgtggatggcgtcgaggtgcacaacgccaaaaccaaaccccgggaggaacagtataacagcacctaccgggtcgtgagcgtgctgaccgtgctgcaccaggattggctgaatggcaaggagtacaagtgcaaggtgtccaacaaagccctgcccgctcccatcgagaagacaatctccaaggccaaaggccagcctcgggaaccccaggtgtataccctcccccccagcagggacgaactgaccaaaaaccaggtgagcctgacctgcctggtgaagggattctaccctagcgatatcgccgtggaatgggagagcaatggacagcctgagaacaactacaaaaccaccccccctgtgctcgactccgatggttctttcttcctgtacagcaaactgaccgtggacaagagccggtggcagcagggcaacgtgttttcctgcagcgtgatgcatgaggctctgcacaaccattacacccagaagagcctgagcctgtcccctggcaagtga

SEQ ID NO: 139 - protein, 475 aa, Artificial Sequence
  GERMLINED 1-85 IgG1 HEAVY CHAIN + YTE
MEWSWVFLFFLSVTTGVHSEVQLVESGGGLVKPGGSLRLSCAASGFTFSDYYMAWIRQAPGKGLEWVSFISSSGRTIYYADSVKGRFTISRDNAKNSLYLQMNSLRAEDTAVYYCARDSYSKLVDIEAIEAFDIWGRGTMVTVSSASTKGPSVFPLAPSSKSTSGGTAALGCLVKDYFPEPVTVSWNSGALTSGVHTFPAVLQSSGLYSLSSVVTVPSSSLGTQTYICNVNHKPSNTKVDKKVEPKSCDKTHTCPPCPAPELLGGPSVFLFPPKPKDTLYITREPEVTCVVVDVSHEDPEVKFNWYVDGVEVHNAKTKPREEQYNSTYRVVSVLTVLHQDWLNGKEYKCKVSNKALPAPIEKTISKAKGQPREPQVYTLPPSRDELTKNQVSLTCLVKGFYPSDIAVEWESNGQPENNYKTTPPVLDSDGSFFLYSKLTVDKSRWQQGNVFSCSVMHEALHNHYTQKSLSLSPGK

SEQ ID NO: 140 - DNA, 705 bp, Artificial Sequence
  GERMLINED 1-85 IgG1 LIGHT CHAIN + YTE
atgtccgtgcccacacaggtgctgggcctgctgctgctgtggctgaccgatgccaggtgctcctacgtgctgacccagcctccttccgtgtccgtggctcctggcaagacagctaggatcacctgcggcggcgacaacatcggcagcaagagcgtgcactggtatcaacagaagcccggccaggcccctgtgctggtgatctactacgattccgaccggcctagcggcatccccgagaggttcagcggctccaactccggcaacaccgccacactgaccatctcccgggtggaggccggagatgaggctgactacttctgccaggtgtgggacaggcatggcgatcacgtggtgttcggcggcggcaccaagctgacagtgctgggacagcctaaggccgctccctccgtgaccctgttcccccctagctccgaggagctgcaggccaacaaggccaccctggtgtgtctcatcagcgacttctaccccggcgctgtgaccgtggcctggaaggctgacagctcccccgtgaaggctggcgtggagaccacaaccccctccaagcagtccaacaataagtacgccgccagctcctacctgtccctgacccccgagcagtggaagagccaccggtcctacagctgccaggtgacccacgaaggctccaccgtggagaagaccgtggcccctaccgagtgcagctga

SEQ ID NO: 141 - protein, 234 aa, Artificial Sequence
  GERMLINED 1-85 IgG1 LIGHT CHAIN + YTE
MSVPTQVLGLLLLWLTDARCSYELAQPPSVSVAPGKTATIACGGDNIGGKSVHWYLQKAGQAPVLVISYDSDRPSGIPERFSGSNSGNTATLTISRVEAGDEADYFCQVWDRHGDHVVFGGGTKLTVLGQPKAAPSVTLFPPSSEELQANKATLVCLISDFYPGAVTVAWKADSSPVKAGVETTTPSKQSNNKYAASSYLSLTPEQWKSHRSYSCQVTHEGSTVEKTVAPTECS

SEQ ID NO: 142 - DNA, 1365 bp, Artificial Sequence
  GERMLINED 3-25 HEAVY CHAIN
caggtgcagctggtggagagcggaggaggagtggtgcagccaggcaggtctctgaggctgagctgcgccgcctccggcttcaccttttccaaccacggcctgcactgggtgcggcaggcacctggcaagggcctggagtgggtggcagtggtgtccaaggacggcacaaatgagcactacgccgattctgtgcggggcagattcaccatctctagggacaacagcaagaatacactgtatctgcagatgaactctctgcgcgccgaggataccgccgtgtactattgtgcccgggagggctactgcggcgacgatagatgttacagcggacagccagactattggggacagggcaccctggtgaccgtgagcagcgcatccaccaagggcccatctgtcttccccctggccccatcctccaagagcacctctggcggcacagctgccctgggctgcctggtgaaggactacttccctgagcctgtgacagtgtcctggaactctggcgccctgaccagcggcgtgcacaccttccctgctgtgctccagtcctctggcctgtactccctgagcagcgtggtgacagtgccatccagcagcctgggcacccagacctacatctgcaatgtgaaccacaagcccagcaacaccaaggtggacaagcgggtggagcccaagtcctgtgacaagacccacacctgccccccatgccccgcccctgagctgctgggcggcccatctgtcttcctgttcccccccaagcccaaggacaccctgatgatctcccggacccccgaggtgacctgtgtggtggtggatgtgagccatgaggaccccgaggtgaagttcaactggtatgtggatggcgtggaggtgcacaacgccaagaccaagccccgggaggagcagtacaacagcacctaccgggtggtgagcgtgctgacagtgctgcatcaggactggctgaatggcaaggagtacaagtgcaaggtgtccaacaaggccctgcctgcccccattgagaagaccatctccaaggccaagggccagccccgggagccccaggtctacaccctgcccccctcccgggaggagatgaccaagaaccaggtgagcctgacctgcctggtgaagggcttctaccccagcgacattgctgtggagtgggagagcaacggccagcctgagaacaactacaagaccaccccccctgtgctggactctgatggctccttcttcctgtacagcaagctgacagtggacaagagccggtggcagcagggcaatgtcttctcctgctctgtgatgcatgaggccctgcacaaccactacacccagaagagcctgtccctgtcccccggcaag

SEQ ID NO: 143 - protein, 455 aa, Artificial Sequence
  GERMLINED 3-25 HEAVY CHAIN
QVQLVESGGGVVQPGRSLRLSCAASGFTFSNHGLHWVRQAPGKGLEWVAVVSKDGTNEHYADSVRGRFTISRDNSKNTLYLQMNSLRAEDTAVYYCAREGYCGDDRCYSGQPDYWGQGTLVTVSSASTKGPSVFPLAPSSKSTSGGTAALGCLVKDYFPEPVTVSWNSGALTSGVHTFPAVLQSSGLYSLSSVVTVPSSSLGTQTYICNVNHKPSNTKVDKRVEPKSCDKTHTCPPCPAPELLGGPSVFLFPPKPKDTLMISRTPEVTCVVVDVSHEDPEVKFNWYVDGVEVHNAKTKPREEQYNSTYRVVSVLTVLHQDWLNGKEYKCKVSNKALPAPIEKTISKAKGQPREPQVYTLPPSREEMTKNQVSLTCLVKGFYPSDIAVEWESNGQPENNYKTTPPVLDSDGSFFLYSKLTVDKSRWQQGNVFSCSVMHEALHNHYTQKSLSLSPGK

SEQ ID NO: 144 - DNA, 645 bp, Artificial Sequence
  GERMLINED 3-25 LIGHT CHAIN
gagatcgtgctgacccagtctcctgccacactgtccctgtctccaggagagagggccaccctgagctgcagagccagccagtccgtgggcagatacctggcctggtatcagcagaagccaggacaggcaccaaggctgctgatctacgacagctccaacagggcaaccggcgtgcccgcacgcttctctggcagcggctccggcacagactttaccctgacaatctctagcctggagcctgaggatttcgccgtgtactattgtcagcagcggtcccactggccacctctgacctttggcggaggcacaaaggtggagatcaagcgtacggtggctgcaccatctgtcttcatcttcccgccatctgatgagcagttgaaatctggaactgcctctgttgtgtgcctgctgaataacttctatcccagagaggccaaagtacagtggaaggtggataacgccctccaatcgggtaactcccaggagagtgtcacagagcaggacagcaaggacagcacctacagcctcagcagcaccctgacgctgagcaaagcagactacgagaaacacaaagtctacgcctgcgaagtcacccatcagggcctgagctcgcccgtcacaaagagcttcaacaggggagagtgt

SEQ ID NO: 145 - protein, 215 aa, Artificial Sequence
  GERMLINED 3-25 LIGHT CHAIN
EIVLTQSPATLSLSPGERATLSCRASQSVGRYLAWYQQKPGQAPRLLIYDSSNRATGVPARFSGSGSGTDFTLTISSLEPEDFAVYYCQQRSHWPPLTFGGGTKVEIKRTVAAPSVFIFPPSDEQLKSGTASVVCLLNNFYPREAKVQWKVDNALQSGNSQESVTEQDSKDSTYSLSSTLTLSKADYEKHKVYACEVTHQGLSSPVTKSFNRGEC

SEQ ID NO: 146 - DNA, 1425 bp, Artificial Sequence
  GERMLINED 3-25 HEAVY CHAIN + YTE
atggaatggagctgggtgttcctgttcttcctgagcgtcaccaccggcgtgcactccgaagtgcagctggtggaatccggcggcggagtcgtgcaacccggcaggtccctgaggctgagctgcgctgcctccggcttcaccttctccaaccatggcctgcactgggtgaggcaagctcccggaaagggcctggagtgggtggctgtcgtgtccaaggacggaaccaacgaacactacgccgactccgtgaggggaaggttcacaatcagccgggacaacagcaagaacacactctatctgcagatgaacagcctgcgggccgaggacacagccgtctactactgcgcccgggaaggatactgcggcgacgataggtgttactccggccagcctgactactggggacagggcaccctggtgaccgtgagcagcgcttccaccaagggccccagcgtgttccctctggctcccagcagcaaatccaccagcggaggcacagctgccctcggatgtctcgtgaaggactattttcccgagcccgtgaccgtctcctggaactctggcgccctgacaagcggcgtgcacacattccccgctgtgctgcagagcagcggactgtattccctgtccagcgtcgtgaccgtcccttcctccagcctgggaacacagacctacatctgcaacgtgaaccacaagccctccaatacaaaggtggacaagaaggtggagcccaagagctgtgacaaaacccatacctgccctccttgccctgctcccgaactgctgggaggaccctccgtctttctgttcccccccaaacccaaggacaccctctacattaccagggagcccgaggtgacctgcgtggtcgtggatgtgagccacgaagatcctgaggtgaagttcaattggtacgtggacggcgtcgaggtgcacaacgccaagaccaagcctcgggaagagcagtacaactccacatacagggtggtgtccgtcctgaccgtcctgcaccaggactggctcaacggcaaggagtacaagtgcaaggtgagcaacaaggccctccccgctcctatcgagaagaccatctccaaggccaaaggacagccccgggagccccaagtgtacaccctgcctccttcccgggatgagctgaccaagaaccaagtctccctgacctgcctcgtgaaaggcttctaccctagcgatatcgctgtggaatgggagtccaacggccagcccgagaataactacaagacaacccctcccgtgctggactccgacggcagcttcttcctgtacagcaagctgaccgtggacaaaagcaggtggcagcagggaaacgtgttctcctgctccgtcatgcacgaggccctgcacaaccactatacccagaagtccctgagcctgtcccccggcaagtga

SEQ ID NO: 147 - protein, 474 aa, Artificial Sequence
  GERMLINED 3-25 HEAVY CHAIN + YTE
MEWSWVFLFFLSVTTGVHSEVQLVESGGGVVQPGRSLRLSCAASGFTFSNHGLHWVRQAPGKGLEWVAVVSKDGTNEHYADSVRGRFTISRDNSKNTLYLQMNSLRAEDTAVYYCAREGYCGDDRCYSGQPDYWGQGTLVTVSSASTKGPSVFPLAPSSKSTSGGTAALGCLVKDYFPEPVTVSWNSGALTSGVHTFPAVLQSSGLYSLSSVVTVPSSSLGTQTYICNVNHKPSNTKVDKKVEPKSCDKTHTCPPCPAPELLGGPSVFLFPPKPKDTLYITREPEVTCVVVDVSHEDPEVKFNWYVDGVEVHNAKTKPREEQYNSTYRVVSVLTVLHQDWLNGKEYKCKVSNKALPAPIEKTISKAKGQPREPQVYTLPPSRDELTKNQVSLTCLVKGFYPSDIAVEWESNGQPENNYKTTPPVLDSDGSFFLYSKLTVDKSRWQQGNVFSCSVMHEALHNHYTQKSLSLSPGK

SEQ ID NO: 148 - DNA, 708 bp, Artificial Sequence
  GERMLINED 3-25 LIGHT CHAIN + YTE
atgtccgtgcccacccaggtgctgggactgctgctgctgtggctgaccgacgccaggtgcgagatcgtgctgacccagagccctgctacactgtccctgagccccggcgagagggctacactgagctgtagggctagccagtccgtgggacggtacctggcctggtaccagcaaaaacccggacaggccccccggctgctgatttacgatagcagcaacagggccaccggcgtgcctgctaggttctccggttctggcagcggcaccgactttaccctgacaatctcctccctggagcccgaggacttcgccgtgtactactgccagcagaggtcccattggcctcctctgaccttcggcggcggcaccaaggtggagatcaagaggaccgtggccgccccctccgtgttcatctttcccccctccgacgagcagctgaagagcggcaccgctagcgtggtgtgcctgctgaacaacttctaccccagggaggccaaggtgcagtggaaggtggacaacgctctgcagtccggcaacagccaggagagcgtgaccgagcaggacagcaaggactccacctactccctgagcagcaccctgaccctgtccaaagccgactacgagaagcacaaggtgtacgcttgcgaggtgacccaccagggcctgtccagccctgtgaccaaatccttcaacaggggcgagtgctga

SEQ ID NO: 149 - protein, 235 aa, Artificial Sequence
  GERMLINED 3-25 LIGHT CHAIN + YTE
MSVPTQVLGLLLLWLTDARCEIVLTQSPATLSLSPGERATLSCRASQSVGRYLAWYQQKPGQAPRLLIYDSSNRATGVPARFSGSGSGTDFTLTISSLEPEDFAVYYCQQRSHWPPLTFGGGTKVEIKRTVAAPSVFIFPPSDEQLKSGTASVVCLLNNFYPREAKVQWKVDNALQSGNSQESVTEQDSKDSTYSLSSTLTLSKADYEKHKVYACEVTHQGLSSPVTKSFNRGEC